European Patent Application EP 4 455 266 A1, published October 30, 2024. Title: 靶向GPRC5D的全人源抗体和嵌合抗原受体(CAR)及其应用. Applicant: 上海驯鹿生物技术有限公司. The sequence listing filed with the application follows.

SEQUENCE LISTING (41 sequences)

SEQ ID NO: 1 - protein, 8 aa, synthetic construct
  REGION 1..8: note = #18 CDR1
GGSFSGYY

SEQ ID NO: 2 - protein, 7 aa, synthetic construct
  REGION 1..7: note = #18 CDR2
INHSGST

SEQ ID NO: 3 - protein, 14 aa, synthetic construct
  REGION 1..14: note = #18 CDR3
ARARRYGGRTRFDP

SEQ ID NO: 4 - protein, 8 aa, synthetic construct
  REGION 1..8: note = #39 CDR1
GFIFSSYG

SEQ ID NO: 5 - protein, 8 aa, synthetic construct
  REGION 1..8: note = #39 CDR2
ISSSGDYT

SEQ ID NO: 6 - protein, 10 aa, synthetic construct
  REGION 1..10: note = #39 CDR3
ARMSFRRYDH

SEQ ID NO: 7 - protein, 8 aa, synthetic construct
  REGION 1..8: note = #41 CDR1
GFSFSGYI

SEQ ID NO: 8 - protein, 8 aa, synthetic construct
  REGION 1..8: note = #41 CDR2
TSSSGTET

SEQ ID NO: 9 - protein, 15 aa, synthetic construct
  REGION 1..15: note = #41 CDR3
ARYYSKYGRSYHVDS

SEQ ID NO: 10 - protein, 120 aa, synthetic construct
  REGION 1..120: note = #18 VHH
QVQLQQWGAGLLKPSETLSLTCAVYGGSFSGYYWSWIRQPPGKGLEWIGEINHSGSTNYNPSLKSRVTISVDTSKNQFSLKLSSVTAADTAVYYCARARRYGGRTRFDPWGQGTLVTVSS

SEQ ID NO: 11 - protein, 117 aa, synthetic construct
  REGION 1..117: note = #39 VHH
EVQLLESGGGLVQPGGSLRLSCAASGFIFSSYGMGWVRQAPGKGLEWVSSISSSGDYTYYADSVKGRFTISRDNSKNTLYLQMNSLRAEDTAVYYCARMSFRRYDHWGQGTLVTVSS

SEQ ID NO: 12 - protein, 122 aa, synthetic construct
  REGION 1..122: note = #41 VHH
EVQLLESGGGLVQPGGSLRLSCAASGFSFSGYIMGWVRQAPGKGLEWVSSTSSSGTETYYADSVKGRFTISRDNSKNTLYLQMNSLRAEDTAVYYCARYYSKYGRSYHVDSWGQGTLVTVSS

SEQ ID NO: 13 - DNA, 360 bp, synthetic construct
  misc_feature 1..360: note = #18 VHH
  source 1..360: mol_type = other DNA
caggtgcagctacagcagtggggcgcaggactgttgaagccttcggagaccctgtccctcacctgcgctgtctatggtgggtccttcagtggttactactggagctggatccgccagcccccagggaaggggctggagtggattggggaaatcaatcatagtggaagcaccaactacaacccgtccctcaagagtcgagtcaccatatcagtagacacgtccaagaaccagttctccctgaagctgagctctgtgaccgccgcggacacggctgtgtattactgtgcgagggcccgacgctacggtggccgaaccaggttcgacccctggggccagggaaccctggtcaccgtctcctca

SEQ ID NO: 14 - DNA, 351 bp, synthetic construct
  misc_feature 1..351: note = #39 VHH
  source 1..351: mol_type = other DNA
gaagttcagctgctggaaagcggtggtggtctggttcagcctggtggtagcctgcgtctgagctgtgcagcaagcggttttatctttagcagctatggcatgggttgggttcgtcaggcacctggtaaaggtctggaatgggttagcagcatcagcagcagcggcgattatacctattatgcagatagcgttaaaggtcgttttaccattagccgtgataacagcaaaaataccctgtacctgcagatgaatagtctgcgtgcagaggataccgcagtgtattattgtgcgcgcatgtctttccgtcgttacgatcattggggtcaaggtactctggtgaccgtctcctca

SEQ ID NO: 15 - DNA, 366 bp, synthetic construct
  misc_feature 1..366: note = #41 VHH
  source 1..366: mol_type = other DNA
gaagttcagctgctggaaagcggtggtggtctggttcagcctggtggtagcctgcgtctgagctgtgcagcaagcggttttagctttagcggctatatcatgggttgggttcgtcaggcacctggtaaaggtctggaatgggttagcagcaccagcagcagcggcaccgaaacctattatgcagatagcgttaaaggtcgttttaccattagccgtgataacagcaaaaataccctgtacctgcagatgaatagtctgcgtgcagaggataccgcagtgtattattgtgcgcgctactactctaaatacggtcgttcttaccatgttgattcttggggtcaaggtactctggtgaccgtctcctca

SEQ ID NO: 16 - DNA, 63 bp, synthetic construct
  misc_feature 1..63: note = CD8 63 bp
  source 1..63: mol_type = other DNA
atggccctgcctgtgacagctctgctcctccctctggccctgctgctccatgccgccagaccc

SEQ ID NO: 17 - protein, 21 aa, synthetic construct
  REGION 1..21: note = CD8 21 aa
MALPVTALLLPLALLLHAARP

SEQ ID NO: 18 - DNA, 165 bp, synthetic construct
  misc_feature 1..165: note = CD8 165 bp
  source 1..165: mol_type = other DNA
ttcgtgcccgtgttcctgcccgccaaacctactactacccctgcacctaggcctcccaccccagccccaacaatcgccagccagcctctgtctctgcggcccgaagcctgtagacctgctgccggcggagccgtgcacaccagaggcctggacttcgcctgcgac

SEQ ID NO: 19 - protein, 55 aa, synthetic construct
  REGION 1..55: note = CD8 55 aa
FVPVFLPAKPTTTPAPRPPTPAPTIASQPLSLRPEACRPAAGGAVHTRGLDFACD

SEQ ID NO: 20 - DNA, 84 bp, synthetic construct
  misc_feature 1..84: note = CD8 84 bp
  source 1..84: mol_type = other DNA
atctacatctgggcccctctggccggcacctgtggcgtgctgctgctgagcctggtgatcaccctgtactgcaaccaccggaac

SEQ ID NO: 21 - protein, 28 aa, synthetic construct
  REGION 1..28: note = CD8 28 aa
IYIWAPLAGTCGVLLLSLVITLYCNHRN

SEQ ID NO: 22 - DNA, 126 bp, synthetic construct
  misc_feature 1..126: note = 4-1BB 126 bp
  source 1..126: mol_type = other DNA
aaacggggcagaaagaaactcctgtatatattcaaacaaccatttatgagaccagtacaaactactcaagaggaagatggctgtagctgccgatttccagaagaagaagaaggaggatgtgaactg

SEQ ID NO: 23 - protein, 42 aa, synthetic construct
  REGION 1..42: note = 4-1BB 42 aa
KRGRKKLLYIFKQPFMRPVQTTQEEDGCSCRFPEEEEGGCEL

SEQ ID NO: 24 - DNA, 336 bp, synthetic construct
  misc_feature 1..336: note = CD3 336 bp
  source 1..336: mol_type = other DNA
agagtgaagttcagcagatccgccgacgcccctgcctaccagcagggacagaaccagctgtacaacgagctgaacctgggcagacgggaagagtacgacgtgctggacaagcggagaggccgggaccccgagatgggcggaaagcccagacggaagaacccccaggaaggcctgtataacgaactgcagaaagacaagatggccgaggcctacagcgagatcggcatgaagggcgagcggaggcgcggcaagggccacgatggcctgtaccagggcctgagcaccgccaccaaggacacctacgacgccctgcacatgcaggccctgccccccaga

SEQ ID NO: 25 - protein, 112 aa, synthetic construct
  REGION 1..112: note = CD3 112 aa
RVKFSRSADAPAYQQGQNQLYNELNLGRREEYDVLDKRRGRDPEMGGKPRRKNPQEGLYNELQKDKMAEAYSEIGMKGERRRGKGHDGLYQGLSTATKDTYDALHMQALPPR

SEQ ID NO: 26 - DNA, 54 bp, synthetic construct
  misc_feature 1..54: note = T2A 54 bp
  source 1..54: mol_type = other DNA
gagggaaggggcagcttattaacatgtggcgatgtggaagagaaccccggtccc

SEQ ID NO: 27 - protein, 18 aa, synthetic construct
  REGION 1..18: note = T2A 18 aa
EGRGSLLTCGDVEENPGP

SEQ ID NO: 28 - DNA, 66 bp, synthetic construct
  misc_feature 1..66: note = CSF2RA signal 66 bp
  source 1..66: mol_type = other DNA
atgctgctgctcgtgacctctttactgttatgtgagctgccccaccccgcttttttactgatccct

SEQ ID NO: 29 - protein, 22 aa, synthetic construct
  REGION 1..22: note = CSF2RA signal 22 aa
MLLLVTSLLLCELPHPAFLLIP

SEQ ID NO: 30 - DNA, 1005 bp, synthetic construct
  misc_feature 1..1005: note = EGFRt 1005 bp
  source 1..1005: mol_type = other DNA
cgtaaggtgtgtaacggaatcggcattggcgagttcaaggactctttaagcatcaacgccacaaacatcaagcacttcaagaattgtacctccatcagcggcgatttacacattctccccgtggcttttcgtggcgattccttcacccacaccccccctctggacccccaagagctggacattttaaaaaccgtgaaggagatcaccggctttctgctgatccaagcttggcccgagaatcgtaccgacctccacgccttcgagaatttagagattattcgtggaaggaccaagcagcacggccagttctctttagccgtcgtgtctttaaacattaccagcctcggtttaaggtctttaaaggagattagcgacggcgacgtgatcatctccggcaacaagaacctctgctacgccaacaccatcaactggaagaagctgttcggaaccagcggccaaaagaccaagatcatcagcaatcgtggagagaactcttgtaaggccactggtcaagtttgccacgccctctgtagccccgaaggatgttggggccccgagcctagggactgtgttagctgcagaaacgtgagcagaggcagagagtgtgtggacaaatgcaatttactggaaggagagcctagggagttcgtggagaacagcgaatgtatccagtgccaccccgagtgtttacctcaagccatgaacatcacttgtaccggaaggggccccgataactgcatccaatgcgcccactacatcgacggaccccactgcgtgaaaacttgtcccgccggagtgatgggagagaataacactttagtgtggaagtacgccgacgctggccacgtctgccatctgtgccaccccaactgtacctacggctgcactggtcccggtttagagggatgtcctaccaacggccccaagatcccctccatcgccaccggaatggtgggcgctctgttattactgctggtggtggctctgggcatcggtttattcatg

SEQ ID NO: 31 - protein, 335 aa, synthetic construct
  REGION 1..335: note = EGFRt 335 aa
RKVCNGIGIGEFKDSLSINATNIKHFKNCTSISGDLHILPVAFRGDSFTHTPPLDPQELDILKTVKEITGFLLIQAWPENRTDLHAFENLEIIRGRTKQHGQFSLAVVSLNITSLGLRSLKEISDGDVIISGNKNLCYANTINWKKLFGTSGQKTKIISNRGENSCKATGQVCHALCSPEGCWGPEPRDCVSCRNVSRGRECVDKCNLLEGEPREFVENSECIQCHPECLPQAMNITCTGRGPDNCIQCAHYIDGPHCVKTCPAGVMGENNTLVWKYADAGHVCHLCHPNCTYGCTGPGLEGCPTNGPKIPSIATGMVGALLLLLVVALGIGLFM

SEQ ID NO: 32 - DNA, 57 bp, synthetic construct
  misc_feature 1..57: note = P2A 57 bp
  source 1..57: mol_type = other DNA
gctactaacttcagcctgctgaagcaggctggtgacgtcgaggagaatcctggcccc

SEQ ID NO: 33 - protein, 19 aa, synthetic construct
  REGION 1..19: note = P2A 19 aa
ATNFSLLKQAGDVEENPGP

SEQ ID NO: 34 - DNA, 1134 bp, synthetic construct
  misc_feature 1..1134: note = GPRC5D CAR 2290(#18) 1134bp
  source 1..1134: mol_type = other DNA
atggccctgcctgtgacagctctgctcctccctctggccctgctgctccatgccgccagaccccaggtgcagctacagcagtggggcgcaggactgttgaagccttcggagaccctgtccctcacctgcgctgtctatggtgggtccttcagtggttactactggagctggatccgccagcccccagggaaggggctggagtggattggggaaatcaatcatagtggaagcaccaactacaacccgtccctcaagagtcgagtcaccatatcagtagacacgtccaagaaccagttctccctgaagctgagctctgtgaccgccgcggacacggctgtgtattactgtgcgagggcccgacgctacggtggccgaaccaggttcgacccctggggccagggaaccctggtcaccgtctcctcattcgtgcccgtgttcctgcccgccaaacctactactacccctgcacctaggcctcccaccccagccccaacaatcgccagccagcctctgtctctgcggcccgaagcctgtagacctgctgccggcggagccgtgcacaccagaggcctggacttcgcctgcgacatctacatctgggcccctctggccggcacctgtggcgtgctgctgctgagcctggtgatcaccctgtactgcaaccaccggaacaaacggggcagaaagaaactcctgtatatattcaaacaaccatttatgagaccagtacaaactactcaagaggaagatggctgtagctgccgatttccagaagaagaagaaggaggatgtgaactgagagtgaagttcagcagatccgccgacgcccctgcctaccagcagggacagaaccagctgtacaacgagctgaacctgggcagacgggaagagtacgacgtgctggacaagcggagaggccgggaccccgagatgggcggaaagcccagacggaagaacccccaggaaggcctgtataacgaactgcagaaagacaagatggccgaggcctacagcgagatcggcatgaagggcgagcggaggcgcggcaagggccacgatggcctgtaccagggcctgagcaccgccaccaaggacacctacgacgccctgcacatgcaggccctgccccccaga

SEQ ID NO: 35 - protein, 378 aa, synthetic construct
  REGION 1..378: note = GPRC5D CAR 2290(#18) 378aa
MALPVTALLLPLALLLHAARPQVQLQQWGAGLLKPSETLSLTCAVYGGSFSGYYWSWIRQPPGKGLEWIGEINHSGSTNYNPSLKSRVTISVDTSKNQFSLKLSSVTAADTAVYYCARARRYGGRTRFDPWGQGTLVTVSSFVPVFLPAKPTTTPAPRPPTPAPTIASQPLSLRPEACRPAAGGAVHTRGLDFACDIYIWAPLAGTCGVLLLSLVITLYCNHRNKRGRKKLLYIFKQPFMRPVQTTQEEDGCSCRFPEEEEGGCELRVKFSRSADAPAYQQGQNQLYNELNLGRREEYDVLDKRRGRDPEMGGKPRRKNPQEGLYNELQKDKMAEAYSEIGMKGERRRGKGHDGLYQGLSTATKDTYDALHMQALPPR

SEQ ID NO: 36 - DNA, 1125 bp, synthetic construct
  misc_feature 1..1125: note = GPRC5D CAR 2436(#39) 1125bp
  source 1..1125: mol_type = other DNA
atggccctgcctgtgacagctctgctcctccctctggccctgctgctccatgccgccagacccgaagttcagctgctggaaagcggtggtggtctggttcagcctggtggtagcctgcgtctgagctgtgcagcaagcggttttatctttagcagctatggcatgggttgggttcgtcaggcacctggtaaaggtctggaatgggttagcagcatcagcagcagcggcgattatacctattatgcagatagcgttaaaggtcgttttaccattagccgtgataacagcaaaaataccctgtacctgcagatgaatagtctgcgtgcagaggataccgcagtgtattattgtgcgcgcatgtctttccgtcgttacgatcattggggtcaaggtactctggtgaccgtctcctcattcgtgcccgtgttcctgcccgccaaacctactactacccctgcacctaggcctcccaccccagccccaacaatcgccagccagcctctgtctctgcggcccgaagcctgtagacctgctgccggcggagccgtgcacaccagaggcctggacttcgcctgcgacatctacatctgggcccctctggccggcacctgtggcgtgctgctgctgagcctggtgatcaccctgtactgcaaccaccggaacaaacggggcagaaagaaactcctgtatatattcaaacaaccatttatgagaccagtacaaactactcaagaggaagatggctgtagctgccgatttccagaagaagaagaaggaggatgtgaactgagagtgaagttcagcagatccgccgacgcccctgcctaccagcagggacagaaccagctgtacaacgagctgaacctgggcagacgggaagagtacgacgtgctggacaagcggagaggccgggaccccgagatgggcggaaagcccagacggaagaacccccaggaaggcctgtataacgaactgcagaaagacaagatggccgaggcctacagcgagatcggcatgaagggcgagcggaggcgcggcaagggccacgatggcctgtaccagggcctgagcaccgccaccaaggacacctacgacgccctgcacatgcaggccctgccccccaga

SEQ ID NO: 37 - protein, 375 aa, synthetic construct
  REGION 1..375: note = GPRC5D CAR 2436(#39) 375aa
MALPVTALLLPLALLLHAARPEVQLLESGGGLVQPGGSLRLSCAASGFIFSSYGMGWVRQAPGKGLEWVSSISSSGDYTYYADSVKGRFTISRDNSKNTLYLQMNSLRAEDTAVYYCARMSFRRYDHWGQGTLVTVSSFVPVFLPAKPTTTPAPRPPTPAPTIASQPLSLRPEACRPAAGGAVHTRGLDFACDIYIWAPLAGTCGVLLLSLVITLYCNHRNKRGRKKLLYIFKQPFMRPVQTTQEEDGCSCRFPEEEEGGCELRVKFSRSADAPAYQQGQNQLYNELNLGRREEYDVLDKRRGRDPEMGGKPRRKNPQEGLYNELQKDKMAEAYSEIGMKGERRRGKGHDGLYQGLSTATKDTYDALHMQALPPR

SEQ ID NO: 38 - DNA, 1140 bp, synthetic construct
  misc_feature 1..1140: note = GPRC5D CAR 2438(#41) 1140bp
  source 1..1140: mol_type = other DNA
atggccctgcctgtgacagctctgctcctccctctggccctgctgctccatgccgccagacccgaagttcagctgctggaaagcggtggtggtctggttcagcctggtggtagcctgcgtctgagctgtgcagcaagcggttttagctttagcggctatatcatgggttgggttcgtcaggcacctggtaaaggtctggaatgggttagcagcaccagcagcagcggcaccgaaacctattatgcagatagcgttaaaggtcgttttaccattagccgtgataacagcaaaaataccctgtacctgcagatgaatagtctgcgtgcagaggataccgcagtgtattattgtgcgcgctactactctaaatacggtcgttcttaccatgttgattcttggggtcaaggtactctggtgaccgtctcctcattcgtgcccgtgttcctgcccgccaaacctactactacccctgcacctaggcctcccaccccagccccaacaatcgccagccagcctctgtctctgcggcccgaagcctgtagacctgctgccggcggagccgtgcacaccagaggcctggacttcgcctgcgacatctacatctgggcccctctggccggcacctgtggcgtgctgctgctgagcctggtgatcaccctgtactgcaaccaccggaacaaacggggcagaaagaaactcctgtatatattcaaacaaccatttatgagaccagtacaaactactcaagaggaagatggctgtagctgccgatttccagaagaagaagaaggaggatgtgaactgagagtgaagttcagcagatccgccgacgcccctgcctaccagcagggacagaaccagctgtacaacgagctgaacctgggcagacgggaagagtacgacgtgctggacaagcggagaggccgggaccccgagatgggcggaaagcccagacggaagaacccccaggaaggcctgtataacgaactgcagaaagacaagatggccgaggcctacagcgagatcggcatgaagggcgagcggaggcgcggcaagggccacgatggcctgtaccagggcctgagcaccgccaccaaggacacctacgacgccctgcacatgcaggccctgccccccaga

SEQ ID NO: 39 - protein, 380 aa, synthetic construct
  REGION 1..380: note = GPRC5D CAR 2438(#41) 380aa
MALPVTALLLPLALLLHAARPEVQLLESGGGLVQPGGSLRLSCAASGFSFSGYIMGWVRQAPGKGLEWVSSTSSSGTETYYADSVKGRFTISRDNSKNTLYLQMNSLRAEDTAVYYCARYYSKYGRSYHVDSWGQGTLVTVSSFVPVFLPAKPTTTPAPRPPTPAPTIASQPLSLRPEACRPAAGGAVHTRGLDFACDIYIWAPLAGTCGVLLLSLVITLYCNHRNKRGRKKLLYIFKQPFMRPVQTTQEEDGCSCRFPEEEEGGCELRVKFSRSADAPAYQQGQNQLYNELNLGRREEYDVLDKRRGRDPEMGGKPRRKNPQEGLYNELQKDKMAEAYSEIGMKGERRRGKGHDGLYQGLSTATKDTYDALHMQALPPR

SEQ ID NO: 40 - DNA, 732 bp, synthetic construct
  source 1..732: mol_type = other DNA
ggatcccaggtgcagctggtgcagagcggcgccgaggtgaagaagcccggcgccagcgtgaaggtgagctgcaaggccagcggctacagcttcaccggctacaccatgaactgggtgcgccaggcccccggccagggcctggagtggatgggcctgatcaacccctacaacagcgacaccaactacgcccagaagctgcagggccgcgtgaccatgaccaccgacaccagcaccagcaccgcctacatggagctgcgcagcctgcgcagcgacgacaccgccgtgtactactgcgcccgcgtggccctgcgcgtggccctggactactggggccagggcaccctggtgaccgtgagcagcggcggcggcggcagcggcggcggcggcagcggcggcggcggcagcgacatccagatgacccagagccccagcagcctgagcgccagcgtgggcgaccgcgtgaccatcacctgcaaggccagccagaacgtggccacccacgtgggctggtaccagcagaagcccggcaaggcccccaagcgcctgatctacagcgccagctaccgctacagcggcgtgcccagccgcttcagcggcagcggcagcggcaccgagttcaccctgaccatcagcaacctgcagcccgaggacttcgccacctactactgccagcagtacaaccgctacccctacaccttcggccagggcaccaagctggagatcaagtctaga

SEQ ID NO: 41 - protein, 244 aa, synthetic construct
GSQVQLVQSGAEVKKPGASVKVSCKASGYSFTGYTMNWVRQAPGQGLEWMGLINPYNSDTNYAQKLQGRVTMTTDTSTSTAYMELRSLRSDDTAVYYCARVALRVALDYWGQGTLVTVSSGGGGSGGGGSGGGGSDIQMTQSPSSLSASVGDRVTITCKASQNVATHVGWYQQKPGKAPKRLIYSASYRYSGVPSRFSGSGSGTEFTLTISNLQPEDFATYYCQQYNRYPYTFGQGTKLEIKSR